European Patent Application EP 4 248 997 A1, published September 27, 2023. Title: Therapeutic or Prophylactic Agent for COVID=19. Applicant: HIROSHIMA UNIVERSITY TOKYO UNIVERSITY OF PHARMACY & LIFE SCIENCES The University of Tokyo Anenti Therapeutics, Inc. The sequence listing filed with the application follows.

SEQUENCE LISTING (2 sequences)

SEQ ID NO: 1 - RNA, 25 nt, Artificial Sequence
  siRNA
cggcaacagcagcagugguggcaaa

SEQ ID NO: 2 - RNA, 25 nt, Artificial Sequence
  siRNA
gcccuggagcugaucaacggcuaca